European Patent Application EP 4 406 613 A2, published July 31, 2024. Title: IMMUNOGENIC ARGINASE PEPTIDES. Applicant: IO BIOTECH APS. Application EP, filed October 6, 2017. The sequence listing filed with the application follows.

SEQUENCE LISTING (62 sequences)

SEQ ID NO: 1 - protein, 322 aa, Homo sapiens
MSAKSRTIGIIGAPFSKGQPRGGVEEGPTVLRKAGLLEKLKEQECDVKDYGDLPFADIPNDSPFQIVKNPRSVGKASEQLAGKVAEVKKNGRISLVLGGDHSLAIGSISGHARVHPDLGVIWVDAHTDINTPLTTTSGNLHGQPVSFLLKELKGKIPDVPGFSWVTPCISAKDIVYIGLRDVDPGEHYILKTLGIKYFSMTEVDRLGIGKVMEETLSYLLGRKKRPIHLSFDVDGLDPSFTPATGTPVVGGLTYREGLYITEEIYKTGLLSGLDIMEVNPSLGKTPEEVTRTVNTAVAITLACFGLAREGNHKPIDYLNPPK

SEQ ID NO: 2 - protein, 9 aa, synthetic construct
  REGION 1..9: note = Artificial sequence
QLAGKVAEV

SEQ ID NO: 3 - protein, 9 aa, synthetic construct
  REGION 1..9: note = Artificial sequence
LVLGGDHSL

SEQ ID NO: 4 - protein, 9 aa, synthetic construct
  REGION 1..9: note = Artificial sequence
LLKELKGKI

SEQ ID NO: 5 - protein, 9 aa, synthetic construct
  REGION 1..9: note = Artificial sequence
ELKGKIPDV

SEQ ID NO: 6 - protein, 9 aa, synthetic construct
  REGION 1..9: note = Artificial sequence
VMEETLSYL

SEQ ID NO: 7 - protein, 9 aa, synthetic construct
  REGION 1..9: note = Artificial sequence
HLSFDVDGL

SEQ ID NO: 8 - protein, 9 aa, synthetic construct
  REGION 1..9: note = Artificial sequence
SLGKTPEEV

SEQ ID NO: 9 - protein, 9 aa, synthetic construct
  REGION 1..9: note = Artificial sequence
IVYIGLRDV

SEQ ID NO: 10 - protein, 9 aa, synthetic construct
  REGION 1..9: note = Artificial sequence
GLLSGLDIM

SEQ ID NO: 11 - protein, 9 aa, synthetic construct
  REGION 1..9: note = Artificial sequence
DIMEVNPSL

SEQ ID NO: 12 - protein, 10 aa, synthetic construct
  REGION 1..10: note = Artificial sequence
LLSGLDIMEV

SEQ ID NO: 13 - protein, 10 aa, synthetic construct
  REGION 1..10: note = Artificial sequence
NLHGQPVSFL

SEQ ID NO: 14 - protein, 10 aa, synthetic construct
  REGION 1..10: note = Artificial sequence
SLVLGGDHSL

SEQ ID NO: 15 - protein, 10 aa, synthetic construct
  REGION 1..10: note = Artificial sequence
YLLGRKKRPI

SEQ ID NO: 16 - protein, 10 aa, synthetic construct
  REGION 1..10: note = Artificial sequence
VLGGDHSLAI

SEQ ID NO: 17 - protein, 10 aa, synthetic construct
  REGION 1..10: note = Artificial sequence
FLLKELKGKI

SEQ ID NO: 18 - protein, 20 aa, synthetic construct
  REGION 1..20: note = Artificial sequence
MSAKSRTIGIIGAPFSKGQP

SEQ ID NO: 19 - protein, 20 aa, synthetic construct
  REGION 1..20: note = Artificial sequence
IGAPFSKGQPRGGVEEGPTV

SEQ ID NO: 20 - protein, 20 aa, synthetic construct
  REGION 1..20: note = Artificial sequence
RGGVEEGPTVLRKAGLLEKL

SEQ ID NO: 21 - protein, 20 aa, synthetic construct
  REGION 1..20: note = Artificial sequence
LRKAGLLEKLKEQECDVKDY

SEQ ID NO: 22 - protein, 20 aa, synthetic construct
  REGION 1..20: note = Artificial sequence
KEQECDVKDYGDLPFADIPN

SEQ ID NO: 23 - protein, 20 aa, synthetic construct
  REGION 1..20: note = Artificial sequence
GDLPFADIPNDSPFQIVKNP

SEQ ID NO: 24 - protein, 20 aa, synthetic construct
  REGION 1..20: note = Artificial sequence
DSPFQIVKNPRSVGKASEQL

SEQ ID NO: 25 - protein, 20 aa, synthetic construct
  REGION 1..20: note = Artificial sequence
RSVGKASEQLAGKVAEVKKN

SEQ ID NO: 26 - protein, 20 aa, synthetic construct
  REGION 1..20: note = Artificial sequence
AGKVAEVKKNGRISLVLGGD

SEQ ID NO: 27 - protein, 20 aa, synthetic construct
  REGION 1..20: note = Artificial sequence
GRISLVLGGDHSLAIGSISG

SEQ ID NO: 28 - protein, 20 aa, synthetic construct
  REGION 1..20: note = Artificial sequence
HSLAIGSISGHARVHPDLGV

SEQ ID NO: 29 - protein, 20 aa, synthetic construct
  REGION 1..20: note = Artificial sequence
HARVHPDLGVIWVDAHTDIN

SEQ ID NO: 30 - protein, 20 aa, synthetic construct
  REGION 1..20: note = Artificial sequence
IWVDAHTDINTPLTTTSGNL

SEQ ID NO: 31 - protein, 20 aa, synthetic construct
  REGION 1..20: note = Artificial sequence
TPLTTTSGNLHGQPVSFLLK

SEQ ID NO: 32 - protein, 20 aa, synthetic construct
  REGION 1..20: note = Artificial sequence
HGQPVSFLLKELKGKIPDVP

SEQ ID NO: 33 - protein, 20 aa, synthetic construct
  REGION 1..20: note = Artificial sequence
ELKGKIPDVPGFSWVTPCIS

SEQ ID NO: 34 - protein, 20 aa, synthetic construct
  REGION 1..20: note = Artificial sequence
GFSWVTPCISAKDIVYIGLR

SEQ ID NO: 35 - protein, 20 aa, synthetic construct
  REGION 1..20: note = Artificial sequence
AKDIVYIGLRDVDPGEHYIL

SEQ ID NO: 36 - protein, 20 aa, synthetic construct
  REGION 1..20: note = Artificial sequence
DVDPGEHYILKTLGIKYFSM

SEQ ID NO: 37 - protein, 20 aa, synthetic construct
  REGION 1..20: note = Artificial sequence
KTLGIKYFSMTEVDRLGIGK

SEQ ID NO: 38 - protein, 20 aa, synthetic construct
  REGION 1..20: note = Artificial sequence
TEVDRLGIGKVMEETLSYLL

SEQ ID NO: 39 - protein, 20 aa, synthetic construct
  REGION 1..20: note = Artificial sequence
VMEETLSYLLGRKKRPIHLS

SEQ ID NO: 40 - protein, 20 aa, synthetic construct
  REGION 1..20: note = Artificial sequence
GRKKRPIHLSFDVDGLDPSF

SEQ ID NO: 41 - protein, 20 aa, synthetic construct
  REGION 1..20: note = Artificial sequence
FDVDGLDPSFTPATGTPVVG

SEQ ID NO: 42 - protein, 20 aa, synthetic construct
  REGION 1..20: note = Artificial sequence
TPATGTPVVGGLTYREGLYI

SEQ ID NO: 43 - protein, 20 aa, synthetic construct
  REGION 1..20: note = Artificial sequence
GLTYREGLYITEEIYKTGLL

SEQ ID NO: 44 - protein, 20 aa, synthetic construct
  REGION 1..20: note = Artificial sequence
TEEIYKTGLLSGLDIMEVNP

SEQ ID NO: 45 - protein, 20 aa, synthetic construct
  REGION 1..20: note = Artificial sequence
SGLDIMEVNPSLGKTPEEVT

SEQ ID NO: 46 - protein, 20 aa, synthetic construct
  REGION 1..20: note = Artificial sequence
SLGKTPEEVTRTVNTAVAIT

SEQ ID NO: 47 - protein, 20 aa, synthetic construct
  REGION 1..20: note = Artificial sequence
RTVNTAVAITLACFGLAREG

SEQ ID NO: 48 - protein, 22 aa, synthetic construct
  REGION 1..22: note = Artificial sequence
LACFGLAREGNHKPIDYLNPPK

SEQ ID NO: 49 - protein, 20 aa, synthetic construct
  REGION 1..20: note = Artificial sequence
GLYITEEIYKTGLLSGLDIM

SEQ ID NO: 50 - protein, 30 aa, synthetic construct
  REGION 1..30: note = Artificial sequence
GFSWVTPCISAKDIVYIGLRDVDPGEHYIL

SEQ ID NO: 51 - protein, 30 aa, synthetic construct
  REGION 1..30: note = Artificial sequence
DVDPGEHYILKTLGIKYFSMTEVDRLGIGK

SEQ ID NO: 52 - protein, 50 aa, synthetic construct
  REGION 1..50: note = Artificial sequence
GFSWVTPCISAKDIVYIGLRDVDPGEHYILKTLGIKYFSMTEVDRLGIGK

SEQ ID NO: 53 - protein, 8 aa, synthetic construct
  REGION 1..8: note = Artificial sequence
KDIVYIGL

SEQ ID NO: 54 - protein, 8 aa, synthetic construct
  REGION 1..8: note = Artificial sequence
LGIKYFSM

SEQ ID NO: 55 - protein, 20 aa, synthetic construct
  REGION 1..20: note = Artificial sequence
DVDPGEHYIIKTLGIKYFSM

SEQ ID NO: 56 - protein, 20 aa, synthetic construct
  REGION 1..20: note = Artificial sequence
KTLGIKYFSMTEVDKLGIGK

SEQ ID NO: 57 - protein, 50 aa, synthetic construct
  REGION 1..50: note = Artificial sequence
GFSWVTPCISAKDIVYIGLRDVDPGEHYIIKTLGIKYFSMTEVDKLGIGK

SEQ ID NO: 58 - protein, 50 aa, synthetic construct
  REGION 1..50: note = Artificial sequence
GFSWIKPCISSASIVYIGLRDVDPPEHFILKNYDIQYFSMRDIDRLGIQK

SEQ ID NO: 59 - protein, 323 aa, synthetic construct
  REGION 1..323: note = Artificial sequence
MSSKPKSLEIIGAPFSKGQPRGGVEKGPAALRKAGLLEKLKETEYDVRDHGDLAFVDVPNDSSFQIVKNPRSVGKANEELAGVVAEVQKNGRVSVVLGGDHSLAVGSISGHARVHPDLCVIWVDAHTDINTPLTTSSGNLHGQPVSFLLKELKGKFPDVPGFSWVTPCISAKDIVYIGLRDVDPGEHYIIKTLGIKYFSMTEVDKLGIGKVMEETFSYLLGRKKRPIHLSFDVDGLDPAFTPATGTPVLGGLSYREGLYITEEIYKTGLLSGLDIMEVNPTLGKTAEEVKSTVNTAVALTLACFGTQREGNHKPGTDYLKPPK

SEQ ID NO: 60 - protein, 354 aa, synthetic construct
  REGION 1..354: note = Artificial sequence
MSLRGSLSRLLQTRVHSILKKSVHSVAVIGAPFSQGQKRKGVEHGPAAIREAGLMKRLSSLGCHLKDFGDLSFTPVPKDDLYNNLIVNPRSVGLANQELAEVVSRAVSDGYSCVTLGGDHSLAIGTISGHARHCPDLCVVWVDAHADINTPLTTSSGNLHGQPVSFLLRELQDKVPQLPGFSWIKPCISSASIVYIGLRDVDPPEHFILKNYDIQYFSMRDIDRLGIQKVMERTFDLLIGKRQRPIHLSFDIDAFDPTLAPATGTPVVGGLTYREGMYIAEEIHNTGLLSALDLVEVNPQLATSEEEAKTTANLAVDVIASSFGQTREGGHIVYDQLPTPSSPDESENQARVRI

SEQ ID NO: 61 - protein, 318 aa, synthetic construct
  REGION 1..318: note = Artificial sequence
MSAKSRTIGIIGAPFSKGQPRGGVEEGPTVLRAGLLEKLKEQECDVKDYGDLPFADIPNDSPFQIVKNPRSVGKASEQLAGKVAEVKKNGRISLVLGGDHSLAISIGHARVHPDLGVIWVDAHTDINTPLTTTSGNLHGQPVSFLLKELKGKIPDVPGFSWVTPCISAKDIVYIGLRDVDPGEHYILKTLGIKYFSMTEVDRLGIGKVMEETLSYLLGRKRPIHLSFDVDGLDPSFTPATGTPVVGGLTYREGLYITEEIYKTGLLSGLDIMEVNPSLGKTPEEVTRTVNTAVAITLACFGLAREGNHKPIDYLNPPK

SEQ ID NO: 62 - protein, 8 aa, synthetic construct
  REGION 1..8: note = Artificial sequence
VTQNFLIL